European Patent Specification EP 3 986 920 B1, published April 16, 2025. Title: TNFR2 antagonists with improved stability. Applicant: University Stuttgart. The sequence listing filed with the application follows.

SEQUENCE LISTING (108 sequences)

SEQ ID NO: 1 - protein, 6 aa, Homo sapiens
  MISC_FEATURE (2)..(2): can be F or Y
  MISC_FEATURE (5)..(5): can be A or I
  MISC_FEATURE (6)..(6): can be a non-polar/hydrophobic or polar/neutral amino acid
VXFGXX

SEQ ID NO: 2 - protein, 5 aa, Homo sapiens
  MISC_FEATURE (2)..(2): can be V or A
  MISC_FEATURE (5)..(5): can be V or L
PXAHX

SEQ ID NO: 3 - protein, 6 aa, Homo sapiens
VYFGII

SEQ ID NO: 4 - protein, 5 aa, Homo sapiens
PVAHV

SEQ ID NO: 5 - protein, 233 aa, Homo sapiens
MSTESMIRDVELAEEALPKKTGGPQGSRRCLFLSLFSFLIVAGATTLFCLLHFGVIGPQREEFPRDLSLISPLAQAVRSSSRTPSDKPVAHVVANPQAEGQLQWLNRRANALLANGVELRDNQLVVPSEGLYLIYSQVLFKGQGCPSTHVLLTHTISRIAVSYQTKVNLLSAIKSPCQRETPEGAEAKPWYEPIYLGGVFQLEKGDRLSAEINRPDYLDFAESGQVYFGIIAL

SEQ ID NO: 6 - protein, 4 aa, Homo sapiens
PSDK

SEQ ID NO: 7 - protein, 5 aa, Homo sapiens
TPSDK

SEQ ID NO: 8 - protein, 6 aa, Homo sapiens
RTPSDK

SEQ ID NO: 9 - protein, 7 aa, Homo sapiens
SRTPSDK

SEQ ID NO: 10 - protein, 8 aa, Homo sapiens
SSRTPSDK

SEQ ID NO: 11 - protein, 4 aa, Homo sapiens
HSTK

SEQ ID NO: 12 - protein, 5 aa, Homo sapiens
AHSTK

SEQ ID NO: 13 - protein, 6 aa, Homo sapiens
LAHSTK

SEQ ID NO: 14 - protein, 7 aa, Homo sapiens
HLAHSTK

SEQ ID NO: 15 - protein, 8 aa, Homo sapiens
LHLAHSTK

SEQ ID NO: 16 - protein, 4 aa, Artificial Sequence
  linker
GGGG

SEQ ID NO: 17 - protein, 4 aa, Artificial Sequence
  linker
GGGS

SEQ ID NO: 18 - protein, 4 aa, Artificial Sequence
  linker
GGSG

SEQ ID NO: 19 - protein, 4 aa, Artificial Sequence
  linker
GSGG

SEQ ID NO: 20 - protein, 4 aa, Artificial Sequence
  linker
SGGG

SEQ ID NO: 21 - protein, 5 aa, Artificial Sequence
  linker
GGGGG

SEQ ID NO: 22 - protein, 5 aa, Artificial Sequence
  linker
SGGGG

SEQ ID NO: 23 - protein, 5 aa, Artificial Sequence
  linker
GSGGG

SEQ ID NO: 24 - protein, 5 aa, Artificial Sequence
  linker
GGSGG

SEQ ID NO: 25 - protein, 5 aa, Artificial Sequence
  linker
GGGSG

SEQ ID NO: 26 - protein, 5 aa, Artificial Sequence
  linker
GGGGS

SEQ ID NO: 27 - protein, 6 aa, Artificial Sequence
  linker
GGGGGG

SEQ ID NO: 28 - protein, 6 aa, Artificial Sequence
  linker
SGGGGG

SEQ ID NO: 29 - protein, 6 aa, Artificial Sequence
  linker
GSGGGG

SEQ ID NO: 30 - protein, 6 aa, Artificial Sequence
  linker
GGSGGG

SEQ ID NO: 31 - protein, 6 aa, Artificial Sequence
  linker
GGGSGG

SEQ ID NO: 32 - protein, 6 aa, Artificial Sequence
  linker
GGGGSG

SEQ ID NO: 33 - protein, 6 aa, Artificial Sequence
  linker
GGGGGS

SEQ ID NO: 34 - protein, 8 aa, Artificial Sequence
  linker
GGGSGGGS

SEQ ID NO: 35 - protein, 8 aa, Artificial Sequence
  linker
SGGGSGGG

SEQ ID NO: 36 - protein, 8 aa, Artificial Sequence
  linker
GGGGGGGG

SEQ ID NO: 37 - protein, 8 aa, Artificial Sequence
  linker
GSGGGSGG

SEQ ID NO: 38 - protein, 8 aa, Artificial Sequence
  linker
GGSGGGSG

SEQ ID NO: 39 - protein, 9 aa, Artificial Sequence
  linker
SGGGSGGGS

SEQ ID NO: 40 - protein, 9 aa, Artificial Sequence
  linker
GSGGGSGGG

SEQ ID NO: 41 - protein, 9 aa, Artificial Sequence
  linker
GGSGGGSGG

SEQ ID NO: 42 - protein, 9 aa, Artificial Sequence
  linker
GGGSGGGSG

SEQ ID NO: 43 - protein, 10 aa, Artificial Sequence
  linker
SGGGSGGGSG

SEQ ID NO: 44 - protein, 10 aa, Artificial Sequence
  linker
GSGGGSGGGS

SEQ ID NO: 45 - protein, 10 aa, Artificial Sequence
  linker
GGSGGGSGGG

SEQ ID NO: 46 - protein, 10 aa, Artificial Sequence
  linker
GGGSGGGSGG

SEQ ID NO: 47 - protein, 11 aa, Artificial Sequence
  linker
SGGGSGGGSGG

SEQ ID NO: 48 - protein, 11 aa, Artificial Sequence
  lnker
GSGGGSGGGSG

SEQ ID NO: 49 - protein, 11 aa, Artificial Sequence
  linker
GGSGGGSGGGS

SEQ ID NO: 50 - protein, 11 aa, Artificial Sequence
  linker
GGGSGGGSGGG

SEQ ID NO: 51 - protein, 9 aa, Homo sapiens
SSSRTPSDK

SEQ ID NO: 52 - protein, 10 aa, Homo sapiens
RSSSRTPSDK

SEQ ID NO: 53 - protein, 12 aa, Artificial Sequence
  linker
GGGSGGGSGGGS

SEQ ID NO: 54 - protein, 16 aa, Artificial Sequence
  linker
GGGSGGGSGGGSGGGS

SEQ ID NO: 55 - protein, 205 aa, Homo sapiens
MTPPERLFLPRVCGTTLHLLLLGLLLVLLPGAQGLPGVGLTPSAAQTARQHPKMHLAHSTLKPAAHLIGDPSKQNSLLWRANTDRAFLQDGFSLSNNSLLVPTSGIYFVYSQVVFSGKAYSPKATSSPLYLAHEVQLFSSQYPFHVPLLSSQKMVYPGLQEPWLHSMYHGAAFQLTQGDQLSTHTDGIPHLVLSPSTVFFGAFAL

SEQ ID NO: 56 - protein, 6 aa, Homo sapiens
VFFGAF

SEQ ID NO: 57 - protein, 5 aa, Homo sapiens
PAAHL

SEQ ID NO: 58 - protein, 23 aa, Artificial Sequence
  scTNFR2 construct
GIIALGGGGSSSRTPSDKPVAHV

SEQ ID NO: 59 - protein, 18 aa, Artificial Sequence
  scTNFR2 construct
GIIALSSRTPSDKPVAHV

SEQ ID NO: 60 - protein, 16 aa, Artificial Sequence
  scTNFR2 contruct
GIIALRTPSDKPVAHV

SEQ ID NO: 61 - protein, 14 aa, Artificial Sequence
  scTNFR2 construct
GIIALPSDKPVAHV

SEQ ID NO: 62 - protein, 17 aa, Artificial Sequence
  scTNFR2 construct
GIIALGGGGSDKPVAHV

SEQ ID NO: 63 - protein, 12 aa, Artificial Sequence
  scTNFR2 construct
GIIALDKPVAHV

SEQ ID NO: 64 - protein, 18 aa, Artificial Sequence
  scTNFR2 construct
GIIALGGGSGGGSPVAHV

SEQ ID NO: 65 - protein, 507 aa, Artificial Sequence
  scTNFR2 (118)
METDTLLLWVLLLWVPGSTGMCGSHHHHHHSGIPASSRTPSDKPVAHVVANPQAEGQLQWLNRRANALLANGVELRDNQLVVPSEGLYLIYSQVLFKGQGCPSTHVLLTHTISRIAVSYQTKVNLLSAIKSPCQRETPEGAEAKPWYEPIYLGGVFQLEKGDRLSAEINRPDYLNFRESGQVYFGIIALGGGGSSSRTPSDKPVAHVVANPQAEGQLQWLNRRANALLANGVELRDNQLVVPSEGLYLIYSQVLFKGQGCPSTHVLLTHTISRIAVSYQTKVNLLSAIKSPCQRETPEGAEAKPWYEPIYLGGVFQLEKGDRLSAEINRPDYLNFRESGQVYFGIIALGGGGSSSRTPSDKPVAHVVANPQAEGQLQWLNRRANALLANGVELRDNQLVVPSEGLYLIYSQVLFKGQGCPSTHVLLTHTISRIAVSYQTKVNLLSAIKSPCQRETPEGAEAKPWYEPIYLGGVFQLEKGDRLSAEINRPDYLNFRESGQVYFGIIAL

SEQ ID NO: 66 - protein, 497 aa, Artificial Sequence
  scTNFR2 (127)
METDTLLLWVLLLWVPGSTGMCGSHHHHHHSGIPASSRTPSDKPVAHVVANPQAEGQLQWLNRRANALLANGVELRDNQLVVPSEGLYLIYSQVLFKGQGCPSTHVLLTHTISRIAVSYQTKVNLLSAIKSPCQRETPEGAEAKPWYEPIYLGGVFQLEKGDRLSAEINRPDYLNFRESGQVYFGIIALSSRTPSDKPVAHVVANPQAEGQLQWLNRRANALLANGVELRDNQLVVPSEGLYLIYSQVLFKGQGCPSTHVLLTHTISRIAVSYQTKVNLLSAIKSPCQRETPEGAEAKPWYEPIYLGGVFQLEKGDRLSAEINRPDYLNFRESGQVYFGIIALSSRTPSDKPVAHVVANPQAEGQLQWLNRRANALLANGVELRDNQLVVPSEGLYLIYSQVLFKGQGCPSTHVLLTHTISRIAVSYQTKVNLLSAIKSPCQRETPEGAEAKPWYEPIYLGGVFQLEKGDRLSAEINRPDYLNFRESGQVYFGIIAL

SEQ ID NO: 67 - protein, 485 aa, Artificial Sequence
  scTNFR2 (129)
METDTLLLWVLLLWVPGSTGMCGSHHHHHHSGIPAPSDKPVAHVVANPQAEGQLQWLNRRANALLANGVELRDNQLVVPSEGLYLIYSQVLFKGQGCPSTHVLLTHTISRIAVSYQTKVNLLSAIKSPCQRETPEGAEAKPWYEPIYLGGVFQLEKGDRLSAEINRPDYLNFRESGQVYFGIIALPSDKPVAHVVANPQAEGQLQWLNRRANALLANGVELRDNQLVVPSEGLYLIYSQVLFKGQGCPSTHVLLTHTISRIAVSYQTKVNLLSAIKSPCQRETPEGAEAKPWYEPIYLGGVFQLEKGDRLSAEINRPDYLNFRESGQVYFGIIALPSDKPVAHVVANPQAEGQLQWLNRRANALLANGVELRDNQLVVPSEGLYLIYSQVLFKGQGCPSTHVLLTHTISRIAVSYQTKVNLLSAIKSPCQRETPEGAEAKPWYEPIYLGGVFQLEKGDRLSAEINRPDYLNFRESGQVYFGIIAL

SEQ ID NO: 68 - protein, 490 aa, Artificial Sequence
  scTNFR2 (139)
METDTLLLWVLLLWVPGSTGMCGSHHHHHHSGIPASDKPVAHVVANPQAEGQLQWLNRRANALLANGVELRDNQLVVPSEGLYLIYSQVLFKGQGCPSTHVLLTHTISRIAVSYQTKVNLLSAIKSPCQRETPEGAEAKPWYEPIYLGGVFQLEKGDRLSAEINRPDYLNFRESGQVYFGIIALGGGGSDKPVAHVVANPQAEGQLQWLNRRANALLANGVELRDNQLVVPSEGLYLIYSQVLFKGQGCPSTHVLLTHTISRIAVSYQTKVNLLSAIKSPCQRETPEGAEAKPWYEPIYLGGVFQLEKGDRLSAEINRPDYLNFRESGQVYFGIIALGGGGSDKPVAHVVANPQAEGQLQWLNRRANALLANGVELRDNQLVVPSEGLYLIYSQVLFKGQGCPSTHVLLTHTISRIAVSYQTKVNLLSAIKSPCQRETPEGAEAKPWYEPIYLGGVFQLEKGDRLSAEINRPDYLNFRESGQVYFGIIAL

SEQ ID NO: 69 - protein, 489 aa, Artificial Sequence
  scTNFR2 (138)
METDTLLLWVLLLWVPGSTGMCGSHHHHHHSGIPAPVAHVVANPQAEGQLQWLNRRANALLANGVELRDNQLVVPSEGLYLIYSQVLFKGQGCPSTHVLLTHTISRIAVSYQTKVNLLSAIKSPCQRETPEGAEAKPWYEPIYLGGVFQLEKGDRLSAEINRPDYLNFRESGQVYFGIIALGGGSGGGSPVAHVVANPQAEGQLQWLNRRANALLANGVELRDNQLVVPSEGLYLIYSQVLFKGQGCPSTHVLLTHTISRIAVSYQTKVNLLSAIKSPCQRETPEGAEAKPWYEPIYLGGVFQLEKGDRLSAEINRPDYLNFRESGQVYFGIIALGGGSGGGSPVAHVVANPQAEGQLQWLNRRANALLANGVELRDNQLVVPSEGLYLIYSQVLFKGQGCPSTHVLLTHTISRIAVSYQTKVNLLSAIKSPCQRETPEGAEAKPWYEPIYLGGVFQLEKGDRLSAEINRPDYLNFRESGQVYFGIIAL

SEQ ID NO: 70 - protein, 491 aa, Artificial Sequence
  scTNFR2 (130)
METDTLLLWVLLLWVPGSTGMCGSHHHHHHSGIPARTPSDKPVAHVVANPQAEGQLQWLNRRANALLANGVELRDNQLVVPSEGLYLIYSQVLFKGQGCPSTHVLLTHTISRIAVSYQTKVNLLSAIKSPCQRETPEGAEAKPWYEPIYLGGVFQLEKGDRLSAEINRPDYLNFRESGQVYFGIIALRTPSDKPVAHVVANPQAEGQLQWLNRRANALLANGVELRDNQLVVPSEGLYLIYSQVLFKGQGCPSTHVLLTHTISRIAVSYQTKVNLLSAIKSPCQRETPEGAEAKPWYEPIYLGGVFQLEKGDRLSAEINRPDYLNFRESGQVYFGIIALRTPSDKPVAHVVANPQAEGQLQWLNRRANALLANGVELRDNQLVVPSEGLYLIYSQVLFKGQGCPSTHVLLTHTISRIAVSYQTKVNLLSAIKSPCQRETPEGAEAKPWYEPIYLGGVFQLEKGDRLSAEINRPDYLNFRESGQVYFGIIAL

SEQ ID NO: 71 - protein, 479 aa, Artificial Sequence
  scTNFR2 (131)
METDTLLLWVLLLWVPGSTGMCGSHHHHHHSGIPADKPVAHVVANPQAEGQLQWLNRRANALLANGVELRDNQLVVPSEGLYLIYSQVLFKGQGCPSTHVLLTHTISRIAVSYQTKVNLLSAIKSPCQRETPEGAEAKPWYEPIYLGGVFQLEKGDRLSAEINRPDYLNFRESGQVYFGIIALDKPVAHVVANPQAEGQLQWLNRRANALLANGVELRDNQLVVPSEGLYLIYSQVLFKGQGCPSTHVLLTHTISRIAVSYQTKVNLLSAIKSPCQRETPEGAEAKPWYEPIYLGGVFQLEKGDRLSAEINRPDYLNFRESGQVYFGIIALDKPVAHVVANPQAEGQLQWLNRRANALLANGVELRDNQLVVPSEGLYLIYSQVLFKGQGCPSTHVLLTHTISRIAVSYQTKVNLLSAIKSPCQRETPEGAEAKPWYEPIYLGGVFQLEKGDRLSAEINRPDYLNFRESGQVYFGIIAL

SEQ ID NO: 72 - protein, 728 aa, Artificial Sequence
  scTNFR2(118)-Fc(dab) 745
METDTLLLWVLLLWVPGSTGSSRTPSDKPVAHVVANPQAEGQLQWLNRRANALLANGVELRDNQLVVPSEGLYLIYSQVLFKGQGCPSTHVLLTHTISRIAVSYQTKVNLLSAIKSPCQRETPEGAEAKPWYEPIYLGGVFQLEKGDRLSAEINRPDYLNFRESGQVYFGIIALGGGGSSSRTPSDKPVAHVVANPQAEGQLQWLNRRANALLANGVELRDNQLVVPSEGLYLIYSQVLFKGQGCPSTHVLLTHTISRIAVSYQTKVNLLSAIKSPCQRETPEGAEAKPWYEPIYLGGVFQLEKGDRLSAEINRPDYLNFRESGQVYFGIIALGGGGSSSRTPSDKPVAHVVANPQAEGQLQWLNRRANALLANGVELRDNQLVVPSEGLYLIYSQVLFKGQGCPSTHVLLTHTISRIAVSYQTKVNLLSAIKSPCQRETPEGAEAKPWYEPIYLGGVFQLEKGDRLSAEINRPDYLNFRESGQVYFGIIALGGSGGGGSGGDKTHTCPPCPAPPVAGPSVFLFPPKPKDTLMISRTPEVTCVVVDVSHEDPEVKFNWYVDGVEVHNAKTKPREEQYNSTYRVVSVLTVLHQDWLNGKEYKCKVSNKGLPSSIEKTISKAKGQPREPQVYTLPPSRDELTKNQVSLTCLVKGFYPSDIAVEWESNGQPENNYKTTPPVLDSDGSFFLYSKLTVDKSRWQQGNVFSCSVMHEALHNHYTQKSLSLSPGK

SEQ ID NO: 73 - protein, 718 aa, Artificial Sequence
  scTNFR2(127)-Fc(dab) 742
METDTLLLWVLLLWVPGSTGSSRTPSDKPVAHVVANPQAEGQLQWLNRRANALLANGVELRDNQLVVPSEGLYLIYSQVLFKGQGCPSTHVLLTHTISRIAVSYQTKVNLLSAIKSPCQRETPEGAEAKPWYEPIYLGGVFQLEKGDRLSAEINRPDYLNFRESGQVYFGIIALSSRTPSDKPVAHVVANPQAEGQLQWLNRRANALLANGVELRDNQLVVPSEGLYLIYSQVLFKGQGCPSTHVLLTHTISRIAVSYQTKVNLLSAIKSPCQRETPEGAEAKPWYEPIYLGGVFQLEKGDRLSAEINRPDYLNFRESGQVYFGIIALSSRTPSDKPVAHVVANPQAEGQLQWLNRRANALLANGVELRDNQLVVPSEGLYLIYSQVLFKGQGCPSTHVLLTHTISRIAVSYQTKVNLLSAIKSPCQRETPEGAEAKPWYEPIYLGGVFQLEKGDRLSAEINRPDYLNFRESGQVYFGIIALGGSGGGGSGGDKTHTCPPCPAPPVAGPSVFLFPPKPKDTLMISRTPEVTCVVVDVSHEDPEVKFNWYVDGVEVHNAKTKPREEQYNSTYRVVSVLTVLHQDWLNGKEYKCKVSNKGLPSSIEKTISKAKGQPREPQVYTLPPSRDELTKNQVSLTCLVKGFYPSDIAVEWESNGQPENNYKTTPPVLDSDGSFFLYSKLTVDKSRWQQGNVFSCSVMHEALHNHYTQKSLSLSPGK

SEQ ID NO: 74 - protein, 706 aa, Artificial Sequence
  scTNFR2(129)-Fc(dab) 743
METDTLLLWVLLLWVPGSTGPSDKPVAHVVANPQAEGQLQWLNRRANALLANGVELRDNQLVVPSEGLYLIYSQVLFKGQGCPSTHVLLTHTISRIAVSYQTKVNLLSAIKSPCQRETPEGAEAKPWYEPIYLGGVFQLEKGDRLSAEINRPDYLNFRESGQVYFGIIALPSDKPVAHVVANPQAEGQLQWLNRRANALLANGVELRDNQLVVPSEGLYLIYSQVLFKGQGCPSTHVLLTHTISRIAVSYQTKVNLLSAIKSPCQRETPEGAEAKPWYEPIYLGGVFQLEKGDRLSAEINRPDYLNFRESGQVYFGIIALPSDKPVAHVVANPQAEGQLQWLNRRANALLANGVELRDNQLVVPSEGLYLIYSQVLFKGQGCPSTHVLLTHTISRIAVSYQTKVNLLSAIKSPCQRETPEGAEAKPWYEPIYLGGVFQLEKGDRLSAEINRPDYLNFRESGQVYFGIIALGGSGGGGSGGDKTHTCPPCPAPPVAGPSVFLFPPKPKDTLMISRTPEVTCVVVDVSHEDPEVKFNWYVDGVEVHNAKTKPREEQYNSTYRVVSVLTVLHQDWLNGKEYKCKVSNKGLPSSIEKTISKAKGQPREPQVYTLPPSRDELTKNQVSLTCLVKGFYPSDIAVEWESNGQPENNYKTTPPVLDSDGSFFLYSKLTVDKSRWQQGNVFSCSVMHEALHNHYTQKSLSLSPGK

SEQ ID NO: 75 - protein, 711 aa, Artificial Sequence
  scTNFR2(139)-Fc(dab) 744
METDTLLLWVLLLWVPGSTGSDKPVAHVVANPQAEGQLQWLNRRANALLANGVELRDNQLVVPSEGLYLIYSQVLFKGQGCPSTHVLLTHTISRIAVSYQTKVNLLSAIKSPCQRETPEGAEAKPWYEPIYLGGVFQLEKGDRLSAEINRPDYLNFRESGQVYFGIIALGGGGSDKPVAHVVANPQAEGQLQWLNRRANALLANGVELRDNQLVVPSEGLYLIYSQVLFKGQGCPSTHVLLTHTISRIAVSYQTKVNLLSAIKSPCQRETPEGAEAKPWYEPIYLGGVFQLEKGDRLSAEINRPDYLNFRESGQVYFGIIALGGGGSDKPVAHVVANPQAEGQLQWLNRRANALLANGVELRDNQLVVPSEGLYLIYSQVLFKGQGCPSTHVLLTHTISRIAVSYQTKVNLLSAIKSPCQRETPEGAEAKPWYEPIYLGGVFQLEKGDRLSAEINRPDYLNFRESGQVYFGIIALGGSGGGGSGGDKTHTCPPCPAPPVAGPSVFLFPPKPKDTLMISRTPEVTCVVVDVSHEDPEVKFNWYVDGVEVHNAKTKPREEQYNSTYRVVSVLTVLHQDWLNGKEYKCKVSNKGLPSSIEKTISKAKGQPREPQVYTLPPSRDELTKNQVSLTCLVKGFYPSDIAVEWESNGQPENNYKTTPPVLDSDGSFFLYSKLTVDKSRWQQGNVFSCSVMHEALHNHYTQKSLSLSPGK

SEQ ID NO: 76 - protein, 495 aa, Artificial Sequence
  variant 140
METDTLLLWVLLLWVPGSTGMCGSHHHHHHSGIPASSRTPSDKPVAHVVANPQAEGQLQWLNRRANALLANGVELRDNQLVVPSEGLYLIYSQVLFKGQGCPSTHVLLTHTISRIAVSYQTKVNLLSAIKSPCQRETPEGAEAKPWYEPIYLGGVFQLEKGDRLSAEINRPDYLNFRESGQVYFGIIALSRTPSDKPVAHVVANPQAEGQLQWLNRRANALLANGVELRDNQLVVPSEGLYLIYSQVLFKGQGCPSTHVLLTHTISRIAVSYQTKVNLLSAIKSPCQRETPEGAEAKPWYEPIYLGGVFQLEKGDRLSAEINRPDYLNFRESGQVYFGIIALSRTPSDKPVAHVVANPQAEGQLQWLNRRANALLANGVELRDNQLVVPSEGLYLIYSQVLFKGQGCPSTHVLLTHTISRIAVSYQTKVNLLSAIKSPCQRETPEGAEAKPWYEPIYLGGVFQLEKGDRLSAEINRPDYLNFRESGQVYFGIIAL

SEQ ID NO: 77 - protein, 497 aa, Artificial Sequence
  variant 141
METDTLLLWVLLLWVPGSTGMCGSHHHHHHSGIPASSRTPSDKPVAHVVANPQAEGQLQWLNRRANALLANGVELRDNQLVVPSEGLYLIYSQVLFKGQGCPSTHVLLTHTISRIAVSYQTKVNLLSAIKSPCQRETPEGAEAKPWYEPIYLGGVFQLEKGDRLSAEINRPDYLNFRESGQVYFGIIALGSRTPSDKPVAHVVANPQAEGQLQWLNRRANALLANGVELRDNQLVVPSEGLYLIYSQVLFKGQGCPSTHVLLTHTISRIAVSYQTKVNLLSAIKSPCQRETPEGAEAKPWYEPIYLGGVFQLEKGDRLSAEINRPDYLNFRESGQVYFGIIALGSRTPSDKPVAHVVANPQAEGQLQWLNRRANALLANGVELRDNQLVVPSEGLYLIYSQVLFKGQGCPSTHVLLTHTISRIAVSYQTKVNLLSAIKSPCQRETPEGAEAKPWYEPIYLGGVFQLEKGDRLSAEINRPDYLNFRESGQVYFGIIAL

SEQ ID NO: 78 - protein, 495 aa, Artificial Sequence
  variant 142
METDTLLLWVLLLWVPGSTGMCGSHHHHHHSGIPASSRTPSDKPVAHVVANPQAEGQLQWLNRRANALLANGVELRDNQLVVPSEGLYLIYSQVLFKGQGCPSTHVLLTHTISRIAVSYQTKVNLLSAIKSPCQRETPEGAEAKPWYEPIYLGGVFQLEKGDRLSAEINRPDYLNFRESGQVYFGIIALGRTPSDKPVAHVVANPQAEGQLQWLNRRANALLANGVELRDNQLVVPSEGLYLIYSQVLFKGQGCPSTHVLLTHTISRIAVSYQTKVNLLSAIKSPCQRETPEGAEAKPWYEPIYLGGVFQLEKGDRLSAEINRPDYLNFRESGQVYFGIIALGRTPSDKPVAHVVANPQAEGQLQWLNRRANALLANGVELRDNQLVVPSEGLYLIYSQVLFKGQGCPSTHVLLTHTISRIAVSYQTKVNLLSAIKSPCQRETPEGAEAKPWYEPIYLGGVFQLEKGDRLSAEINRPDYLNFRESGQVYFGIIAL

SEQ ID NO: 79 - protein, 490 aa, Artificial Sequence
  variant 143
METDTLLLWVLLLWVPGSTGMCGSHHHHHHSGIPASDKPVAHVVANPQAEGQLQWLNRRANALLANGVELRDNQLVVPSEGLYLIYSQVLFKGQGCPSTHVLLTHTISRIAVSYQTKVNLLSAIKSPCQRETPEGAEAKPWYEPIYLGGVFQLEKGDRLSAEINRPDYLNFRESGQVYFGIIALGGGPSDKPVAHVVANPQAEGQLQWLNRRANALLANGVELRDNQLVVPSEGLYLIYSQVLFKGQGCPSTHVLLTHTISRIAVSYQTKVNLLSAIKSPCQRETPEGAEAKPWYEPIYLGGVFQLEKGDRLSAEINRPDYLNFRESGQVYFGIIALGGGPSDKPVAHVVANPQAEGQLQWLNRRANALLANGVELRDNQLVVPSEGLYLIYSQVLFKGQGCPSTHVLLTHTISRIAVSYQTKVNLLSAIKSPCQRETPEGAEAKPWYEPIYLGGVFQLEKGDRLSAEINRPDYLNFRESGQVYFGIIAL

SEQ ID NO: 80 - protein, 497 aa, Artificial Sequence
  variant 144
METDTLLLWVLLLWVPGSTGMCGSHHHHHHSGIPASSRTPSDKPVAHVVANPQAEGQLQWLNRRANALLANGVELRDNQLVVPSEGLYLIYSQVLFKGQGCPSTHVLLTHTISRIAVSYQTKVNLLSAIKSPCQRETPEGAEAKPWYEPIYLGGVFQLEKGDRLSAEINRPDYLNFRESGQVYFGIIALGGRTPSDKPVAHVVANPQAEGQLQWLNRRANALLANGVELRDNQLVVPSEGLYLIYSQVLFKGQGCPSTHVLLTHTISRIAVSYQTKVNLLSAIKSPCQRETPEGAEAKPWYEPIYLGGVFQLEKGDRLSAEINRPDYLNFRESGQVYFGIIALGGRTPSDKPVAHVVANPQAEGQLQWLNRRANALLANGVELRDNQLVVPSEGLYLIYSQVLFKGQGCPSTHVLLTHTISRIAVSYQTKVNLLSAIKSPCQRETPEGAEAKPWYEPIYLGGVFQLEKGDRLSAEINRPDYLNFRESGQVYFGIIAL

SEQ ID NO: 81 - protein, 493 aa, Artificial Sequence
  variant 145
METDTLLLWVLLLWVPGSTGMCGSHHHHHHSGIPARTPSDKPVAHVVANPQAEGQLQWLNRRANALLANGVELRDNQLVVPSEGLYLIYSQVLFKGQGCPSTHVLLTHTISRIAVSYQTKVNLLSAIKSPCQRETPEGAEAKPWYEPIYLGGVFQLEKGDRLSAEINRPDYLNFRESGQVYFGIIALGGTPSDKPVAHVVANPQAEGQLQWLNRRANALLANGVELRDNQLVVPSEGLYLIYSQVLFKGQGCPSTHVLLTHTISRIAVSYQTKVNLLSAIKSPCQRETPEGAEAKPWYEPIYLGGVFQLEKGDRLSAEINRPDYLNFRESGQVYFGIIALGGTPSDKPVAHVVANPQAEGQLQWLNRRANALLANGVELRDNQLVVPSEGLYLIYSQVLFKGQGCPSTHVLLTHTISRIAVSYQTKVNLLSAIKSPCQRETPEGAEAKPWYEPIYLGGVFQLEKGDRLSAEINRPDYLNFRESGQVYFGIIAL

SEQ ID NO: 82 - protein, 492 aa, Artificial Sequence
  variant 146
METDTLLLWVLLLWVPGSTGMCGSHHHHHHSGIPASDKPVAHVVANPQAEGQLQWLNRRANALLANGVELRDNQLVVPSEGLYLIYSQVLFKGQGCPSTHVLLTHTISRIAVSYQTKVNLLSAIKSPCQRETPEGAEAKPWYEPIYLGGVFQLEKGDRLSAEINRPDYLNFRESGQVYFGIIALGGGTPSDKPVAHVVANPQAEGQLQWLNRRANALLANGVELRDNQLVVPSEGLYLIYSQVLFKGQGCPSTHVLLTHTISRIAVSYQTKVNLLSAIKSPCQRETPEGAEAKPWYEPIYLGGVFQLEKGDRLSAEINRPDYLNFRESGQVYFGIIALGGGTPSDKPVAHVVANPQAEGQLQWLNRRANALLANGVELRDNQLVVPSEGLYLIYSQVLFKGQGCPSTHVLLTHTISRIAVSYQTKVNLLSAIKSPCQRETPEGAEAKPWYEPIYLGGVFQLEKGDRLSAEINRPDYLNFRESGQVYFGIIAL

SEQ ID NO: 83 - protein, 492 aa, Artificial Sequence
  variant 147
METDTLLLWVLLLWVPGSTGMCGSHHHHHHSGIPASDKPVAHVVANPQAEGQLQWLNRRANALLANGVELRDNQLVVPSEGLYLIYSQVLFKGQGCPSTHVLLTHTISRIAVSYQTKVNLLSAIKSPCQRETPEGAEAKPWYEPIYLGGVFQLEKGDRLSAEINRPDYLNFRESGQVYFGIIALGGGGPSDKPVAHVVANPQAEGQLQWLNRRANALLANGVELRDNQLVVPSEGLYLIYSQVLFKGQGCPSTHVLLTHTISRIAVSYQTKVNLLSAIKSPCQRETPEGAEAKPWYEPIYLGGVFQLEKGDRLSAEINRPDYLNFRESGQVYFGIIALGGGGPSDKPVAHVVANPQAEGQLQWLNRRANALLANGVELRDNQLVVPSEGLYLIYSQVLFKGQGCPSTHVLLTHTISRIAVSYQTKVNLLSAIKSPCQRETPEGAEAKPWYEPIYLGGVFQLEKGDRLSAEINRPDYLNFRESGQVYFGIIAL

SEQ ID NO: 84 - protein, 716 aa, Artificial Sequence
  variant 148
METDTLLLWVLLLWVPGSTGSSRTPSDKPVAHVVANPQAEGQLQWLNRRANALLANGVELRDNQLVVPSEGLYLIYSQVLFKGQGCPSTHVLLTHTISRIAVSYQTKVNLLSAIKSPCQRETPEGAEAKPWYEPIYLGGVFQLEKGDRLSAEINRPDYLNFRESGQVYFGIIALSRTPSDKPVAHVVANPQAEGQLQWLNRRANALLANGVELRDNQLVVPSEGLYLIYSQVLFKGQGCPSTHVLLTHTISRIAVSYQTKVNLLSAIKSPCQRETPEGAEAKPWYEPIYLGGVFQLEKGDRLSAEINRPDYLNFRESGQVYFGIIALSRTPSDKPVAHVVANPQAEGQLQWLNRRANALLANGVELRDNQLVVPSEGLYLIYSQVLFKGQGCPSTHVLLTHTISRIAVSYQTKVNLLSAIKSPCQRETPEGAEAKPWYEPIYLGGVFQLEKGDRLSAEINRPDYLNFRESGQVYFGIIALGGSGGGGSGGDKTHTCPPCPAPPVAGPSVFLFPPKPKDTLMISRTPEVTCVVVDVSHEDPEVKFNWYVDGVEVHNAKTKPREEQYNSTYRVVSVLTVLHQDWLNGKEYKCKVSNKGLPSSIEKTISKAKGQPREPQVYTLPPSRDELTKNQVSLTCLVKGFYPSDIAVEWESNGQPENNYKTTPPVLDSDGSFFLYSKLTVDKSRWQQGNVFSCSVMHEALHNHYTQKSLSLSPGK

SEQ ID NO: 85 - protein, 718 aa, Artificial Sequence
  variant 149
METDTLLLWVLLLWVPGSTGSSRTPSDKPVAHVVANPQAEGQLQWLNRRANALLANGVELRDNQLVVPSEGLYLIYSQVLFKGQGCPSTHVLLTHTISRIAVSYQTKVNLLSAIKSPCQRETPEGAEAKPWYEPIYLGGVFQLEKGDRLSAEINRPDYLNFRESGQVYFGIIALGSRTPSDKPVAHVVANPQAEGQLQWLNRRANALLANGVELRDNQLVVPSEGLYLIYSQVLFKGQGCPSTHVLLTHTISRIAVSYQTKVNLLSAIKSPCQRETPEGAEAKPWYEPIYLGGVFQLEKGDRLSAEINRPDYLNFRESGQVYFGIIALGSRTPSDKPVAHVVANPQAEGQLQWLNRRANALLANGVELRDNQLVVPSEGLYLIYSQVLFKGQGCPSTHVLLTHTISRIAVSYQTKVNLLSAIKSPCQRETPEGAEAKPWYEPIYLGGVFQLEKGDRLSAEINRPDYLNFRESGQVYFGIIALGGSGGGGSGGDKTHTCPPCPAPPVAGPSVFLFPPKPKDTLMISRTPEVTCVVVDVSHEDPEVKFNWYVDGVEVHNAKTKPREEQYNSTYRVVSVLTVLHQDWLNGKEYKCKVSNKGLPSSIEKTISKAKGQPREPQVYTLPPSRDELTKNQVSLTCLVKGFYPSDIAVEWESNGQPENNYKTTPPVLDSDGSFFLYSKLTVDKSRWQQGNVFSCSVMHEALHNHYTQKSLSLSPGK

SEQ ID NO: 86 - protein, 711 aa, Artificial Sequence
  variant 150
METDTLLLWVLLLWVPGSTGSDKPVAHVVANPQAEGQLQWLNRRANALLANGVELRDNQLVVPSEGLYLIYSQVLFKGQGCPSTHVLLTHTISRIAVSYQTKVNLLSAIKSPCQRETPEGAEAKPWYEPIYLGGVFQLEKGDRLSAEINRPDYLNFRESGQVYFGIIALGRTPSDKPVAHVVANPQAEGQLQWLNRRANALLANGVELRDNQLVVPSEGLYLIYSQVLFKGQGCPSTHVLLTHTISRIAVSYQTKVNLLSAIKSPCQRETPEGAEAKPWYEPIYLGGVFQLEKGDRLSAEINRPDYLNFRESGQVYFGIIALGRTPSDKPVAHVVANPQAEGQLQWLNRRANALLANGVELRDNQLVVPSEGLYLIYSQVLFKGQGCPSTHVLLTHTISRIAVSYQTKVNLLSAIKSPCQRETPEGAEAKPWYEPIYLGGVFQLEKGDRLSAEINRPDYLNFRESGQVYFGIIALGGSGGGGSGGDKTHTCPPCPAPPVAGPSVFLFPPKPKDTLMISRTPEVTCVVVDVSHEDPEVKFNWYVDGVEVHNAKTKPREEQYNSTYRVVSVLTVLHQDWLNGKEYKCKVSNKGLPSSIEKTISKAKGQPREPQVYTLPPSRDELTKNQVSLTCLVKGFYPSDIAVEWESNGQPENNYKTTPPVLDSDGSFFLYSKLTVDKSRWQQGNVFSCSVMHEALHNHYTQKSLSLSPGK

SEQ ID NO: 87 - protein, 711 aa, Artificial Sequence
  variant 151
METDTLLLWVLLLWVPGSTGSDKPVAHVVANPQAEGQLQWLNRRANALLANGVELRDNQLVVPSEGLYLIYSQVLFKGQGCPSTHVLLTHTISRIAVSYQTKVNLLSAIKSPCQRETPEGAEAKPWYEPIYLGGVFQLEKGDRLSAEINRPDYLNFRESGQVYFGIIALGGGPSDKPVAHVVANPQAEGQLQWLNRRANALLANGVELRDNQLVVPSEGLYLIYSQVLFKGQGCPSTHVLLTHTISRIAVSYQTKVNLLSAIKSPCQRETPEGAEAKPWYEPIYLGGVFQLEKGDRLSAEINRPDYLNFRESGQVYFGIIALGGGPSDKPVAHVVANPQAEGQLQWLNRRANALLANGVELRDNQLVVPSEGLYLIYSQVLFKGQGCPSTHVLLTHTISRIAVSYQTKVNLLSAIKSPCQRETPEGAEAKPWYEPIYLGGVFQLEKGDRLSAEINRPDYLNFRESGQVYFGIIALGGSGGGGSGGDKTHTCPPCPAPPVAGPSVFLFPPKPKDTLMISRTPEVTCVVVDVSHEDPEVKFNWYVDGVEVHNAKTKPREEQYNSTYRVVSVLTVLHQDWLNGKEYKCKVSNKGLPSSIEKTISKAKGQPREPQVYTLPPSRDELTKNQVSLTCLVKGFYPSDIAVEWESNGQPENNYKTTPPVLDSDGSFFLYSKLTVDKSRWQQGNVFSCSVMHEALHNHYTQKSLSLSPGK

SEQ ID NO: 88 - protein, 718 aa, Artificial Sequence
  variant 152
METDTLLLWVLLLWVPGSTGSSRTPSDKPVAHVVANPQAEGQLQWLNRRANALLANGVELRDNQLVVPSEGLYLIYSQVLFKGQGCPSTHVLLTHTISRIAVSYQTKVNLLSAIKSPCQRETPEGAEAKPWYEPIYLGGVFQLEKGDRLSAEINRPDYLNFRESGQVYFGIIALGGRTPSDKPVAHVVANPQAEGQLQWLNRRANALLANGVELRDNQLVVPSEGLYLIYSQVLFKGQGCPSTHVLLTHTISRIAVSYQTKVNLLSAIKSPCQRETPEGAEAKPWYEPIYLGGVFQLEKGDRLSAEINRPDYLNFRESGQVYFGIIALGGRTPSDKPVAHVVANPQAEGQLQWLNRRANALLANGVELRDNQLVVPSEGLYLIYSQVLFKGQGCPSTHVLLTHTISRIAVSYQTKVNLLSAIKSPCQRETPEGAEAKPWYEPIYLGGVFQLEKGDRLSAEINRPDYLNFRESGQVYFGIIALGGSGGGGSGGDKTHTCPPCPAPPVAGPSVFLFPPKPKDTLMISRTPEVTCVVVDVSHEDPEVKFNWYVDGVEVHNAKTKPREEQYNSTYRVVSVLTVLHQDWLNGKEYKCKVSNKGLPSSIEKTISKAKGQPREPQVYTLPPSRDELTKNQVSLTCLVKGFYPSDIAVEWESNGQPENNYKTTPPVLDSDGSFFLYSKLTVDKSRWQQGNVFSCSVMHEALHNHYTQKSLSLSPGK

SEQ ID NO: 89 - protein, 714 aa, Artificial Sequence
  variant 153
METDTLLLWVLLLWVPGSTGRTPSDKPVAHVVANPQAEGQLQWLNRRANALLANGVELRDNQLVVPSEGLYLIYSQVLFKGQGCPSTHVLLTHTISRIAVSYQTKVNLLSAIKSPCQRETPEGAEAKPWYEPIYLGGVFQLEKGDRLSAEINRPDYLNFRESGQVYFGIIALGGTPSDKPVAHVVANPQAEGQLQWLNRRANALLANGVELRDNQLVVPSEGLYLIYSQVLFKGQGCPSTHVLLTHTISRIAVSYQTKVNLLSAIKSPCQRETPEGAEAKPWYEPIYLGGVFQLEKGDRLSAEINRPDYLNFRESGQVYFGIIALGGTPSDKPVAHVVANPQAEGQLQWLNRRANALLANGVELRDNQLVVPSEGLYLIYSQVLFKGQGCPSTHVLLTHTISRIAVSYQTKVNLLSAIKSPCQRETPEGAEAKPWYEPIYLGGVFQLEKGDRLSAEINRPDYLNFRESGQVYFGIIALGGSGGGGSGGDKTHTCPPCPAPPVAGPSVFLFPPKPKDTLMISRTPEVTCVVVDVSHEDPEVKFNWYVDGVEVHNAKTKPREEQYNSTYRVVSVLTVLHQDWLNGKEYKCKVSNKGLPSSIEKTISKAKGQPREPQVYTLPPSRDELTKNQVSLTCLVKGFYPSDIAVEWESNGQPENNYKTTPPVLDSDGSFFLYSKLTVDKSRWQQGNVFSCSVMHEALHNHYTQKSLSLSPGK

SEQ ID NO: 90 - protein, 713 aa, Artificial Sequence
  variant 154
METDTLLLWVLLLWVPGSTGSDKPVAHVVANPQAEGQLQWLNRRANALLANGVELRDNQLVVPSEGLYLIYSQVLFKGQGCPSTHVLLTHTISRIAVSYQTKVNLLSAIKSPCQRETPEGAEAKPWYEPIYLGGVFQLEKGDRLSAEINRPDYLNFRESGQVYFGIIALGGGTPSDKPVAHVVANPQAEGQLQWLNRRANALLANGVELRDNQLVVPSEGLYLIYSQVLFKGQGCPSTHVLLTHTISRIAVSYQTKVNLLSAIKSPCQRETPEGAEAKPWYEPIYLGGVFQLEKGDRLSAEINRPDYLNFRESGQVYFGIIALGGGTPSDKPVAHVVANPQAEGQLQWLNRRANALLANGVELRDNQLVVPSEGLYLIYSQVLFKGQGCPSTHVLLTHTISRIAVSYQTKVNLLSAIKSPCQRETPEGAEAKPWYEPIYLGGVFQLEKGDRLSAEINRPDYLNFRESGQVYFGIIALGGSGGGGSGGDKTHTCPPCPAPPVAGPSVFLFPPKPKDTLMISRTPEVTCVVVDVSHEDPEVKFNWYVDGVEVHNAKTKPREEQYNSTYRVVSVLTVLHQDWLNGKEYKCKVSNKGLPSSIEKTISKAKGQPREPQVYTLPPSRDELTKNQVSLTCLVKGFYPSDIAVEWESNGQPENNYKTTPPVLDSDGSFFLYSKLTVDKSRWQQGNVFSCSVMHEALHNHYTQKSLSLSPGK

SEQ ID NO: 91 - protein, 713 aa, Artificial Sequence
  variant 155
METDTLLLWVLLLWVPGSTGSDKPVAHVVANPQAEGQLQWLNRRANALLANGVELRDNQLVVPSEGLYLIYSQVLFKGQGCPSTHVLLTHTISRIAVSYQTKVNLLSAIKSPCQRETPEGAEAKPWYEPIYLGGVFQLEKGDRLSAEINRPDYLNFRESGQVYFGIIALGGGGPSDKPVAHVVANPQAEGQLQWLNRRANALLANGVELRDNQLVVPSEGLYLIYSQVLFKGQGCPSTHVLLTHTISRIAVSYQTKVNLLSAIKSPCQRETPEGAEAKPWYEPIYLGGVFQLEKGDRLSAEINRPDYLNFRESGQVYFGIIALGGGGPSDKPVAHVVANPQAEGQLQWLNRRANALLANGVELRDNQLVVPSEGLYLIYSQVLFKGQGCPSTHVLLTHTISRIAVSYQTKVNLLSAIKSPCQRETPEGAEAKPWYEPIYLGGVFQLEKGDRLSAEINRPDYLNFRESGQVYFGIIALGGSGGGGSGGDKTHTCPPCPAPPVAGPSVFLFPPKPKDTLMISRTPEVTCVVVDVSHEDPEVKFNWYVDGVEVHNAKTKPREEQYNSTYRVVSVLTVLHQDWLNGKEYKCKVSNKGLPSSIEKTISKAKGQPREPQVYTLPPSRDELTKNQVSLTCLVKGFYPSDIAVEWESNGQPENNYKTTPPVLDSDGSFFLYSKLTVDKSRWQQGNVFSCSVMHEALHNHYTQKSLSLSPGK

SEQ ID NO: 92 - protein, 10 aa, Artificial Sequence
  linker
GGSGGGGSGG

SEQ ID NO: 93 - protein, 18 aa, Artificial Sequence
  from variant 141
GIIALGSRTPSDKPVAHV

SEQ ID NO: 94 - protein, 18 aa, Artificial Sequence
  from variant 144
GIIALGGRTPSDKPVAHV

SEQ ID NO: 95 - protein, 18 aa, Artificial Sequence
  from variant 146
GIIALGGGTPSDKPVAHV

SEQ ID NO: 96 - protein, 18 aa, Artificial Sequence
  from variant 147
GIIALGGGGPSDKPVAHV

SEQ ID NO: 97 - protein, 17 aa, Artificial Sequence
  from variant 140
GIIALSRTPSDKPVAHV

SEQ ID NO: 98 - protein, 17 aa, Artificial Sequence
  from variant 142
GIIALGRTPSDKPVAHV

SEQ ID NO: 99 - protein, 17 aa, Artificial Sequence
  from variant 145
GIIALGGTPSDKPVAHV

SEQ ID NO: 100 - protein, 17 aa, Artificial Sequence
  from variant 143
GIIALGGGPSDKPVAHV

SEQ ID NO: 101 - protein, 18 aa, Artificial Sequence
  from variant 149
GIIALGSRTPSDKPVAHV

SEQ ID NO: 102 - protein, 18 aa, Artificial Sequence
  from variant 152
GIIALGGRTPSDKPVAHV

SEQ ID NO: 103 - protein, 18 aa, Artificial Sequence
  from variant 154
GIIALGGGTPSDKPVAHV

SEQ ID NO: 104 - protein, 18 aa, Artificial Sequence
  from variant 155
GIIALGGGGPSDKPVAHV

SEQ ID NO: 105 - protein, 17 aa, Artificial Sequence
  from variant 148
GIIALSRTPSDKPVAHV

SEQ ID NO: 106 - protein, 17 aa, Artificial Sequence
  from variant 150
GIIALGRTPSDKPVAHV

SEQ ID NO: 107 - protein, 17 aa, Artificial Sequence
  from variant 153
GIIALGGTPSDKPVAHV

SEQ ID NO: 108 - protein, 17 aa, Artificial Sequence
  from variant 151
GIIALGGGPSDKPVAHV